European Patent Application EP 4 488 374 A1, published January 8, 2025. Title: Verfahren zur Herstellung einer wässerigen Lösung enthaltend Ethylenglycol. Applicant: Annikki GmbH. Application EP. The sequence listing filed with the application follows.

SEQUENCE LISTING (8 sequences)

SEQ ID NO: 1 - protein, 337 aa, Geobacillus stearothermophilus
MKAAVVEQFKKPLQVKEVEKPKISYGEVLVRIKACGVCHTDLHAAHGDWPVKPKLPLIPGHEGVGVIEEVGPGVTHLKVGDRVGIPWLYSACGHCDYCLSGQETLCERQQNAGYSVDGGYAEYCRAAADYVVKIPDNLSFEEAAPIFCAGVTTYKALKVTGAKPGEWVAIYGIGGLGHVAVQYAKAMGLNVVAVDLGDEKLELAKQLGADLVVNPKHDDAAQWIKEKVGGVHATVVTAVSKAAFESAYKSIRRGGACVLVGLPPEEIPIPIFDTVLNGVKIIGSIVGTRKDLQEALQFAAEGKVKTIVEVQPLENINDVFDRMLKGQINGRVVLKVD

SEQ ID NO: 2 - DNA, 1014 bp, Geobacillus stearothermophilus
  source 1..1014: mol_type = genomic DNA
atgaaagctgcagttgtggaacaatttaaaaagccgttacaagtgaaagaagtggaaaaacctaagatctcatacggggaagtattagtgcgcatcaaagcgtgtggggtatgccatacagacttgcatgccgcacatggcgactggcctgtaaagcctaaactgcctctcattcctggccatgaaggcgtcggtgtaattgaagaagtaggtcctggggtaacacatttaaaagttggagatcgcgtaggtatcccttggctttattcggcgtgcggtcattgtgactattgcttaagcggacaagaaacattatgcgaacgtcaacaaaacgctggctattccgtcgatggtggttatgctgaatattgccgtgctgcagccgattatgtcgtaaaaattcctgataacttatcgtttgaagaagccgctccaatcttttgcgctggtgtaacaacatataaagcgctcaaagtaacaggcgcaaaaccaggtgaatgggtagccatttacggtatcggcgggcttggacatgtcgcagtccaatacgcaaaggcgatggggttaaacgtcgttgctgtcgatttaggtgatgaaaaacttgagcttgctaaacaacttggtgcagatcttgtcgtcaatccgaaacatgatgatgcagcacaatggataaaagaaaaagtgggcggtgtgcatgcgactgtcgtcacagctgtttcaaaagccgcgttcgaatcagcctacaaatccattcgtcgcggtggtgcttgcgtactcgtcggattaccgccggaagaaatacctattccaattttcgatacagtattaaatggagtaaaaattattggttctatcgttggtacgcgcaaagacttacaagaggcacttcaatttgcagcagaaggaaaagtaaaaacaattgtcgaagtgcaaccgcttgaaaacattaacgacgtattcgatcgtatgttaaaagggcaaattaacggccgcgtcgtgttaaaagtagattaa

SEQ ID NO: 3 - protein, 342 aa, Acetobacter pasteurianus
MSGKMKAAVVHEFGKPLTIEELDIPTIKPTQILVKMIACGVCHTDLHAASGDWPKKPHLPFIPGHEGVGTVVQVGSEVDWVKEGDVVGVPWLYSACGHCEHCLAGWETLCAKQEETGYSVNGCFAEYVVADPNYIAHLPKGVDPVKVAPVLCAGLTVYKGLKMTDTRAGNWVAISGVGGLGQMAVQYAVAMGLNVVAVDIDDEKLATAKKLGATYTVNARNTDPAAFMQEKVGGVHGGLITAVSTKAFSQAMGYVRAGGTLVLNGLPPGDFPISIFDVVMNAITIRGSIVGTRLDMIEALSFFAEGKVTSVTTTDRIDNINAIFDALKNGRVEGRVVLDFRN

SEQ ID NO: 4 - DNA, 1029 bp, Acetobacter pasteurianus
  source 1..1029: mol_type = genomic DNA
atgtccggaaaaatgaaagccgctgtggttcatgaatttggcaaaccactgaccattgaagaactggacattcccaccattaaacccacccagattttggttaaaatgattgcctgcggcgtgtgccatacagatttgcatgctgccagcggggattggcccaaaaaaccacatctgccgtttattcccggccacgaaggcgttggcacggttgtgcaggttggcagcgaagtagactgggtaaaggaaggcgacgttgttggcgtgccttggctctattctgcctgcggccattgcgagcattgtctggctgggtgggaaaccctttgtgcgaagcaagaagaaaccggctattccgtaaacggctgctttgccgaatacgtggtagcagaccctaactacattgctcatcttcccaaaggcgtagaccctgtaaaagttgcccccgtactgtgcgcaggcctgaccgtttataagggcctgaaaatgacagacacgcgggcagggaactgggttgccatttccggcgttggggggttaggccagatggctgtgcagtacgccgtagcaatggggctgaatgttgtggcggtagatattgatgatgaaaaactggcaaccgccaaaaagcttggtgcaacgtacactgttaacgccagaaatacagatccggcagcatttatgcaggaaaaagttggtggcgtacacggtggattgatcaccgctgtttccaccaaagcattttctcaggctatgggttatgtgcgggcagggggcactttggtgctaaatgggctgccgccgggtgatttcccaatttctatctttgacgtggtcatgaatgccattaccattcgcggctccatagtaggcacacggctggacatgattgaagctctttccttctttgcggaagggaaggtaacatctgtcaccacaacggatcggattgataacatcaacgcaatttttgatgcgctcaagaacggtcgggtggaaggccgcgtggttctggacttccgcaactga

SEQ ID NO: 5 - protein, 342 aa, Achromobacter xylosoxidans
MNKTMKAAVARAFGKPLEIEEVEVPRPRAGELLVKIEACGVCHTDLHAVEGDWPVKPNPPFIPGHEGVGHVVAVGEGVTHVKEGDRVGIPWLYSACGHCEHCLGGWETLCEQQQNAGYSVNGGFAEYALAAADYVGLLPKNVGFVDIAPVLCAGVTVYKGLKMTDTRPGNWVVVSGIGGLGHMAVQYARAMGLNVAAVDIDDDKLDFAKRLGAEVVVNAKATDPAAYLKKEIGGAHGALITAVSPKAFEQALGMVRRGGTVALNGLPPGDFPLSIFDMVLNGVTVRGSIVGSRLDLQESLQFAEEGKVRATVATEKLENINSVFDRMRRGQIEGRIVLDMAA

SEQ ID NO: 6 - DNA, 1029 bp, Achromobacter xylosoxidans
  source 1..1029: mol_type = genomic DNA
atgaacaagaccatgaaggccgcggtggcccgcgcgttcggcaaacccctggaaatcgaagaagtcgaggtgccgcgcccgcgcgcgggcgaactgttggtgaagatcgaggcctgcggcgtctgccacaccgatctgcacgcggtcgagggcgactggccggtcaagcccaatccccctttcatcccgggccacgaaggcgtgggccacgtggtggcggtgggcgaaggcgtgacgcacgtcaaggaaggcgaccgcgtcggcatcccctggctgtattccgcctgtggccattgcgagcattgcctgggcggctgggagacgctgtgcgaacagcagcagaacgccggctactccgtcaacggcggcttcgccgagtacgcgctggccgcggccgactacgtgggcctgctgccgaagaatgtcggcttcgtcgacatcgccccggtactgtgcgccggcgtcacggtctacaaaggcctgaagatgacggacacacggccaggcaactgggtcgtggtctccggcatcggcggcctgggccacatggcggtgcagtatgcgcgcgccatgggcttgaacgtggcggccgtggacatcgacgacgacaaactggatttcgccaagcgtctcggcgccgaggtggtcgtgaatgccaaggccaccgatccagcggcttacctgaagaaggaaatcggcggcgcccacggcgcgctgatcacggcggtttcgcccaaggccttcgagcaggcgctgggcatggtgcgtcgcggcggcacggtggcgctcaacggcctgccgccgggcgacttcccgctgtcgatcttcgacatggtgctcaacggcgtgacggtgcgcggttcgatcgtgggttcgcgcctggacttgcaggaatcgctgcagttcgccgaggaaggcaaggtgcgcgcgaccgtggcgaccgagaagctggagaacatcaacagcgtgttcgaccgcatgcgccgcggccagatcgaaggccgcatcgtgctggacatggcggcgtaa

SEQ ID NO: 7 - protein, 324 aa, Candida tropicalis
MSTTVNTPTIKLNSGYEMPLVGFGCWKVTNATAADQIYNAIKTGYRLFDGAEDYGNEKEVGEGINRAIKDGLVKREELFITSKLWNNFHDPKNVETALNKTLSDLNLDYVDLFLIHFPIAFKFVPIEEKYPPGFYCGDGDNFHYEDVPLLDTWKALEKLVEAGKIKSIGISNFTGALIYDLIRGATIKPAVLQIEHHPYLQQPKLIEYVQKAGIAITGYSSFGPQSFLELESKRALNTPTLFEHETIKSIADKHGKSPAQVLLRWATQRNIAVIPKSNNPERLAQNLSVVDFDLTKDDLDNIAKLDIGLRFNDPWDWDNIPIFV

SEQ ID NO: 8 - DNA, 974 bp, Candida tropicalis
  source 1..974: mol_type = genomic DNA
atgagcacgaccgttaatactccgacgatcaaactgaactccggttacgagatgccgctggttggctttggctgttggaaagttaccaatgcgacggcggcggaccagatttataacgctattaaaaccggttaccgtctgttcgatggcgcagaggactacggtaacgagaaagaagtgggtgaaggtattaatcgcgcaattaaagacggtctggtcaaacgtgaagagctgtttattacctcgaaactgtggaataacttccatgatcctaagaacgtggagactgcgctgaataagaccctgagcgatctgaacctggactatgtggatctgtttctgattcacttcccgattgctttcaaatttgtcccgatcgaagaaaagtacccaccgggcttctactgcggtgacggcgacaacttccattatgaggatgttccgctgctggacacgtggaaggcgctggagaaattggtggaagccggtaagatcaagtccattggcattagcaacttcaccggtgccttgatttacgatttgatccgtggtgcgaccattaaaccggcggttctgcagatcgagcatcacccgtatctgcaacagccgaaactgatcgaatacgttcagaaagcaggtatcgccatcactggctatagcagcttcggtccacagagcttcctggagctggagagcaagcgtgccctgaataccccgacgttgtttgaacacgaaaccatcaagtctatcgctgacaaacacggtaagagccctgcacaagtcctgctgcgctgggcaacgcaacgtaatattgcggttattccgaagagcaataacccggagcgtctggcgcagaatctgtctgtcgtcgactttgatttgaccaaggatgacctggataatatcgcgaagctggacatcggcctgcgcttcaacgatccgtgggattgggacaacatcccgatctttgtgta